European Patent Application EP 4 692 354 A1, published February 11, 2026. Title: Recombinant protein. Applicant: Kikkoman Corporation. The sequence listing filed with the application follows.

SEQUENCE LISTING (25 sequences)

SEQ ID NO: 1 - DNA, 24 bp, synthetic construct
  misc_feature 1..24: note = primer
  source 1..24: mol_type = other DNA
tctagagggcccgcggttcgaagg

SEQ ID NO: 2 - DNA, 25 bp, synthetic construct
  misc_feature 1..25: note = primer
  source 1..25: mol_type = other DNA
ggtaccaagctttaaattcgaacag

SEQ ID NO: 3 - protein, 1020 aa, Limulus polyphemus
MVLASFLVSGLVLGLLAQQMHPVQSRGVDLGLCDDTRFECKCGDPGYVFNVPAKQCTYFYRWRPYCKPCDKLEAKDVCPKYKRCQECRAGLDSCVSCPPNKYGTWCSGECQCKNGGICDQRTGACTCRDRYEGVHCEILQGCPLLQSDPQVQEVKNPPNDPQTIDYSCSPGFKLKGVARITCLPNGQWSSFPPKCIRECSMVSSLEHGKVNSPSADLIEGATLRFSCDSPYYLIGQETLTCQGNGQWSGQIPQCQKLVFCPDLDPVSHAEHQVKIGLEQKYGQFPQGTEVTYTCTGNYFLMGLDTLKCNPDGSWSGTQPSCVKVADREVNCDSKAVDFLDDVGEPVRIHCPAGCSLTAGTVWGTAIYHELSSVCRAAIHAGKVPNSGGAVHVVNNGPYSDFLASDLNGIKSDELKSLAQSFRFDYVSSSTAGRKSGCPDGWFEIEENCVYVTSKQRAWERAQGVCTNMAARLAVLDKDVIPSSLTETLRGKGLATTWIGLHRLDADNHFIWELMDRSSVALNDSLTFWAPGEPGNETNCVYLDIQDQLQPVWKTKSCFQPSSFVCMMDLSDKNKAKCKDPGPLENGHAKLHGQSIDGFYAGSSVRYSCEVLHYLSGTETVSCTSNGTWSAPKPRCIKVITCQTPPVPSYGSVDIKPPSRTNSISRVGSPFLRLPRLPLPLARAAGPPPKPRSAPPSTVDLSSKVKLPEGHYRVGSQAIYTCESRYYELLGSQGRRCDSNGKWSGRPASCIPVCGRSDSPRSPFIVNGNSTEIGQWPWQAGISRWLADHNMWFLQCGGALLNEKWIITAAHCVTYSATAEIIDPSQFKFYLGKYYRDDSKDDDYVQVREAIEIHVNPNYDPGNLNFDIALIQLKTSVALTTRVQPICLPTDLTTRENLKEGALAVVTGWGLNENNTYSEMIQQAVLPVVAASTCEQGYQDSGLPLTVTENMFCAGYKQGRYDACSGDSGGPLVFADDSRTDRRWVLEGIVSWGSPNGCGKSNQYGGFTKVNVFLSWIRQFI

SEQ ID NO: 4 - DNA, 3063 bp, Limulus polyphemus
  source 1..3063: mol_type = other DNA
atggtgctggctagcttcctggtgtctggactggtgctgggactgctggctcagcaaatgcaccctgtgcagtctcgtggtgtcgacctgggattgtgcgacgacactcgtttcgagtgcaagtgcggcgaccccggttacgtgttcaacgtgccagctaagcagtgcacctacttctaccgttggcgcccctactgcaagccctgcgacaagttggaagctaaggacgtgtgccccaagtacaagcgttgccaagagtgccgtgctggcctggactcctgtgtttcttgccctcctaacaaatacggcacctggtgctctggcgagtgccagtgcaagaacggtggtatctgcgaccagcgtaccggtgcttgcacttgccgtgatcgttacgagggtgtccactgcgagatcctgcaaggttgccctctgctgcagtctgaccctcaggtgcaagaagtgaagaaccctccaaacgaccctcagaccatcgactactcttgctctcccggtttcaagctgaagggtgtcgctcgtatcacttgcctgcctaacggccagtggtctagcttcccacctaagtgcatccgcgagtgctccatggtgtcctcactcgagcacggcaaagtgaactctccctccgctgacctgatcgagggtgctaccttgaggttctcctgcgactccccttactacctgatcggtcaagagactctgacctgccaaggcaacggacagtggagcggtcaaatccctcagtgccaaaagctggtgttctgccccgacttggaccccgtgtctcacgctgaacaccaagtgaagatcggcctcgagcagaagtacggacagttccctcagggcaccgaagtgacctacacctgtaccggcaactacttcctgatgggcctcgacaccctgaagtgcaaccctgacggttcttggagcggtactcagccctcctgcgtgaaagtggctgaccgtgaagtgaactgcgactctaaggctgtggacttcctggacgacgtgggagagcctgtgcgtattcactgtcctgctggttgctccctgaccgctggtactgtttggggcaccgctatctaccacgagctgtcctctgtgtgccgcgctgctattcacgctggaaaggtgcccaactccggtggtgctgtgcacgtggtcaacaacggtccctactccgacttcctcgcttccgacctgaacggtatcaagtccgacgagctgaagtccctggctcagtccttccgtttcgactacgtgtcctcctccaccgctggacgcaagtctggttgtcctgacggatggttcgagatcgaagagaactgcgtgtacgtgacctccaagcagagagcttgggaacgcgctcaaggcgtgtgcaccaatatggctgctcgtctggctgtgctggacaaggacgtgatcccttccagcctgactgagactctgcgtggaaagggactcgctaccacctggatcggactgcaccgtttggacgctgacaaccacttcatctgggagctgatggaccgttcctccgtggctctgaacgactctctgactttctgggctcctggcgagcctggcaacgagactaactgcgtctacctggacatccaggaccagctgcagcccgtgtggaaaactaagtcctgcttccagccatcctccttcgtgtgcatgatggacctgtccgacaagaacaaggctaagtgcaaggaccccggtcctctcgagaacggtcacgctaagctgcacggccagtccatcgacggtttctacgctggttcctctgtgcgctactcctgcgaggtgctgcactacctgtccggaaccgagactgtgtcctgcacctccaacggaacttggagcgcacctaagcctcgttgcatcaaagtgatcacctgtcagacccctccagtgccttcctacggttccgtggacatcaagccaccttctcgtaccaactccatctctcgtgtgggttctcccttcctgcgtctgcctcgtttgcctctgcctttggctagagctgctggtccacctcctaagccacgttccgctcctccatctaccgtggacttgtcctccaaagtgaagctgcccgagggccactaccgtgtcggttcccaggctatctacacttgcgagtcccgctactacgaactgctgggttctcagggtcgtcgttgcgactcaaatggcaagtggagtggtcgtcccgcttcttgcatccctgtgtgcggtcgttctgactcccctcgttctcctttcatcgtgaacggcaactccaccgagatcggccaatggccttggcaagctggtatctccagatggctggctgaccacaacatgtggttcttgcagtgcggtggcgctctgctgaacgagaagtggatcatcaccgctgctcactgcgtgacctactccgctaccgctgagatcatcgacccctctcagttcaagttctacctgggcaagtactaccgtgacgactccaaggacgacgactacgtccaagtgcgcgaggctatcgagatccacgtgaaccctaactacgaccccggcaacctgaacttcgatatcgctctgatccagctcaagacctctgtcgctctgaccaccagggtgcagcctatctgcttgcctaccgacctgaccactcgcgagaacctgaaagagggtgctctcgctgtcgtgaccggatggggactcaacgagaacaacacctactctgagatgatccagcaggccgtgctgccagtggtggctgcttctacttgcgagcagggttaccaggactccggactgcctctgactgtgaccgaaaacatgttctgcgctggttacaagcagggccgttacgacgcttgctcaggcgattctggtggtcccctggtgttcgctgacgactctcgtactgatcgtcgttgggtgctcgagggtatcgtgtcctggggttctcctaacggttgcggcaagtccaaccagtacggtggttttaccaaagtcaacgtgttcctgtcctggatccgtcagttcatctga

SEQ ID NO: 5 - DNA, 28 bp, synthetic construct
  misc_feature 1..28: note = homologous sequence
  source 1..28: mol_type = other DNA
ctgttcgaatttaaagcttggtaccgat

SEQ ID NO: 6 - DNA, 21 bp, synthetic construct
  misc_feature 1..21: note = homologous sequence
  source 1..21: mol_type = other DNA
tctagagggcccgcggttcga

SEQ ID NO: 7 - DNA, 30 bp, synthetic construct
  misc_feature 1..30: note = primer
  source 1..30: mol_type = other DNA
cagtggtctagcctcccacctaagtgcatc

SEQ ID NO: 8 - DNA, 30 bp, synthetic construct
  misc_feature 1..30: note = primer
  source 1..30: mol_type = other DNA
gctagaccactggccgttaggcaggcaagt

SEQ ID NO: 9 - DNA, 30 bp, synthetic construct
  misc_feature 1..30: note = primer
  source 1..30: mol_type = other DNA
cagtccttccgtctcgactacgtgtcctcc

SEQ ID NO: 10 - DNA, 30 bp, synthetic construct
  misc_feature 1..30: note = primer
  source 1..30: mol_type = other DNA
acggaaggactgagccagggacttcagctc

SEQ ID NO: 11 - DNA, 30 bp, synthetic construct
  misc_feature 1..30: note = primer
  source 1..30: mol_type = other DNA
actaagtcctgcctccagccatcctccttc

SEQ ID NO: 12 - DNA, 30 bp, synthetic construct
  misc_feature 1..30: note = primer
  source 1..30: mol_type = other DNA
gcaggacttagttttccacacgggctgcag

SEQ ID NO: 13 - DNA, 30 bp, synthetic construct
  misc_feature 1..30: note = primer
  source 1..30: mol_type = other DNA
gtgggttctccctacctgcgtctgcctcgt

SEQ ID NO: 14 - DNA, 30 bp, synthetic construct
  misc_feature 1..30: note = primer
  source 1..30: mol_type = other DNA
gggagaacccacacgagagatggagttggt

SEQ ID NO: 15 - DNA, 30 bp, synthetic construct
  misc_feature 1..30: note = primer
  source 1..30: mol_type = other DNA
gtgggttctcccctcctgcgtctgcctcgt

SEQ ID NO: 16 - DNA, 30 bp, synthetic construct
  misc_feature 1..30: note = primer
  source 1..30: mol_type = other DNA
tctcagttcaagctctacctgggcaagtac

SEQ ID NO: 17 - DNA, 30 bp, synthetic construct
  misc_feature 1..30: note = primer
  source 1..30: mol_type = other DNA
cttgaactgagaggggtcgatgatctcagc

SEQ ID NO: 18 - DNA, 30 bp, synthetic construct
  misc_feature 1..30: note = primer
  source 1..30: mol_type = other DNA
tctggtggtcccgcggtgttcgctgacgac

SEQ ID NO: 19 - DNA, 30 bp, synthetic construct
  misc_feature 1..30: note = primer
  source 1..30: mol_type = other DNA
gggaccaccagaatcgcctgagcaagcgtc

SEQ ID NO: 20 - DNA, 30 bp, synthetic construct
  misc_feature 1..30: note = primer
  source 1..30: mol_type = other DNA
tctggtggtcccgtggtgttcgctgacgac

SEQ ID NO: 21 - DNA, 30 bp, synthetic construct
  misc_feature 1..30: note = primer
  source 1..30: mol_type = other DNA
cccctggtgttcttagacgactctcgtact

SEQ ID NO: 22 - DNA, 30 bp, synthetic construct
  misc_feature 1..30: note = primer
  source 1..30: mol_type = other DNA
gaacaccaggggaccaccagaatcgcctga

SEQ ID NO: 23 - DNA, 30 bp, synthetic construct
  misc_feature 1..30: note = primer
  source 1..30: mol_type = other DNA
tccaaccagtactctggttttaccaaagtc

SEQ ID NO: 24 - DNA, 30 bp, synthetic construct
  misc_feature 1..30: note = primer
  source 1..30: mol_type = other DNA
gtactggttggacttgccgcaaccgttagg

SEQ ID NO: 25 - DNA, 30 bp, synthetic construct
  misc_feature 1..30: note = primer
  source 1..30: mol_type = other DNA
tccaaccagtacactggttttaccaaagtc